European Patent Application EP 4 137 155 A1, published February 22, 2023. Title: PREPARATION SPECIFICALLY BOUND WITH CD137 AND USE THEREOF. Applicant: DINGFU BIOTARGET, CO., LTD. The sequence listing filed with the application follows.

SEQUENCE LISTING (36 sequences)

SEQ ID NO: 1 - protein, 111 aa, Artificial Sequence
  C2-4A VL
QSALIQPPSASGSPGQSVTISCTGISSDVGAYDYVSWYQQHPGKVPKLMIYEVSKRPSGVPDRFSGSKSGNTASLTISGLQAEDEADYYCSSHAGSNNFYVFGTGTKLTVL

SEQ ID NO: 2 - protein, 111 aa, Artificial Sequence
  C2-4B VL
QSVLIQPPSVSGSPGQSVTISCTGISSDVGAYDYVSWYQQHPGKVPKLMIYEVSKRPSGVPDRFSGSKSGDTASLTISGLQAEDEADYYCSSHAGSNNFYVFGTGTKLTVL

SEQ ID NO: 3 - protein, 111 aa, Artificial Sequence
  C2-4C VL
QSVLIQPPSASGSPGQSVTISCTGISSDVGAYDYVSWYQQHPGKVPKLMIYEVSKRPSGVPDRFSGSKSGNTASLTVSGLQAEDEADYYCSSHAGSNNFYVFGTGTKLTVL

SEQ ID NO: 4 - protein, 111 aa, Artificial Sequence
  C2-5A VL
QSVLIQPPSVSGSPGQSVTISCTGISSDVGAYDYVSWYQQHPGKVPKLMIYEVSKRPSGVPDRFSGSKSGNTASLTISGLQAEDEADYYCSSHAGSNNFYVFGTGTKLTVL

SEQ ID NO: 5 - protein, 111 aa, Artificial Sequence
  C2-5B VL
QSVLIQPPSASGSPGQSVTISCTGISSDVGAYDYVSWYQQHPGKVPKLMIYEVSKRPSGVPDRFSGSKSGNTASLTISGLQAEDEADYYCSSHAGSNNFYVFGTGTKLTVL

SEQ ID NO: 6 - protein, 111 aa, Artificial Sequence; identical to SEQ ID NO: 2
  C2-5C VL

SEQ ID NO: 7 - protein, 111 aa, Artificial Sequence; identical to SEQ ID NO: 4
  C2-6A VL

SEQ ID NO: 8 - protein, 111 aa, Artificial Sequence
  C2-6B VL
QSVLIQPPSVSGSPGQSVTISCTGISSDVGAYDYVSWYQQHPGKVPKLMIYEVSKRPSGVPDRFSGSKSGNTASLTVSGLQAEDEADYYCSSHAGSNNFYVFGTGTKLTVL

SEQ ID NO: 9 - protein, 111 aa, Artificial Sequence
  C2-7A VL
QSALIQPPSVSGSPGQSVTISCTGISSDVGAYDYVSWYQQHPGTVPKLMIYEVSKRPSGVPDRFSGSKSGNTASLTISGLQAEDEADYYCSSHAGSNNFYVFGTGTKLTVL

SEQ ID NO: 10 - protein, 111 aa, Artificial Sequence; identical to SEQ ID NO: 2
  C2-7B VL

SEQ ID NO: 11 - protein, 111 aa, Artificial Sequence; identical to SEQ ID NO: 2
  C2-7BN78K VL

SEQ ID NO: 12 - protein, 124 aa, Artificial Sequence
  C2-4A VH
EVQLVESGGGLVQPGGSLRLSCAASGFTVSDYYMNWIRQAPGKGLEWVSYISSSASGSTIYYADSVKGRFTISRDNAKNSLYLHMDSLRAEDTAIYFCARVVPAGSGWRWFDPWGQGTLVTVSS

SEQ ID NO: 13 - protein, 124 aa, Artificial Sequence
  C2-4B VH
EVQLVESGGGLVQPGRSLRLSCAASGFTVSDYYMNWFRQAPGKGLEWVSYISSSASGSTIYYADSVKGRFTISRDNANNSLYLHMDSLRAEDTAIYFCARVVPAGSGWRWFDPWGQGTLVTVSS

SEQ ID NO: 14 - protein, 124 aa, Artificial Sequence
  C2-4C VH
EVQLVESGGGLVQPGGSLRLSCAASGFTVSDYYMNWIRQAPGKGLEWVSYISSSASGSTIYYADSVKGRFTISRDNAKNSLYLQMNSLRAEDTAIYFCARVVPAGSGWRWFDPWGQGTLVTVSS

SEQ ID NO: 15 - protein, 124 aa, Artificial Sequence
  C2-5A VH
EVQLVESGGGLVQPGRSLRLSCAASGFTVSDYYMNWIRQAPGKGLEWVSYISSSASGSTIYYADSVKGRFTISRDNAKNSLYLHMDSLRAEDTAIYFCARVVPAGSGWRWFDPWGQGTLVTVSS

SEQ ID NO: 16 - protein, 124 aa, Artificial Sequence; identical to SEQ ID NO: 14
  C2-5B VH

SEQ ID NO: 17 - protein, 124 aa, Artificial Sequence
  C2-5C VH
EVQLVESGGGLVQPGRSLRLSCAASGFTVSDYYMNWFRQAPGKGLEWVSYISSSASGSTIYYADSVKGRFTISRDNANNSLYLHMDSLRAEDTAIYYCARVVPAGSGWRWFDPWGQGTLVTVSS

SEQ ID NO: 18 - protein, 124 aa, Artificial Sequence; identical to SEQ ID NO: 14
  C2-6A VH

SEQ ID NO: 19 - protein, 124 aa, Artificial Sequence
  C2-6B VH
EVQLVESGGGLVKPGGSLRLSCAASGFTVSDYYMNWIRQAPGKGLEWVSYISSSASGSTIYYADSVKGRFTISRDNAKNSLYLQMNSLRAEDTAIYFCARVVPAGSGWRWFDPWGQGTLVTVSS

SEQ ID NO: 20 - protein, 124 aa, Artificial Sequence
  C2-7A VH
EVQLVESGGGLVKPGGSLRLSCAASGFTVSDYYMNWIRQAPGKGLEWVSYISSSASGSTIYYADSVKGRFTISRDNAKNSLYLHMDSLRAEDTAIYFCARVVPAGSGWRWFDPWGQGTLVTVSS

SEQ ID NO: 21 - protein, 124 aa, Artificial Sequence
  C2-7B VH
EVQLVESGGGLVKPGGSLRLSCAASGFTVSDYYMNWIRQAPGKGLEWVSYISSSASGSTIYYADSVKGRFTISRDNANNSLYLQMNSLRTEDTAIYYCARVVPAGSGWRWFDPWGQGTLVTVSS

SEQ ID NO: 22 - protein, 124 aa, Artificial Sequence
  C2-7BN78K VH
EVQLVESGGGLVKPGGSLRLSCAASGFTVSDYYMNWIRQAPGKGLEWVSYISSSASGSTIYYADSVKGRFTISRDNAKNSLYLQMNSLRTEDTAIYYCARVVPAGSGWRWFDPWGQGTLVTVSS

SEQ ID NO: 23 - protein, 484 aa, Artificial Sequence
  C2-4A-Fc
EVQLVESGGGLVQPGGSLRLSCAASGFTVSDYYMNWIRQAPGKGLEWVSYISSSASGSTIYYADSVKGRFTISRDNAKNSLYLHMDSLRAEDTAIYFCARVVPAGSGWRWFDPWGQGTLVTVSSGGGGSGGGGSGGGGSQSALIQPPSASGSPGQSVTISCTGISSDVGAYDYVSWYQQHPGKVPKLMIYEVSKRPSGVPDRFSGSKSGNTASLTISGLQAEDEADYYCSSHAGSNNFYVFGTGTKLTVLGGGGSESKYGPPCPPCPAPEFLGGPSVFLFPPKPKDTLMISRTPEVTCVVVDVSQEDPEVQFNWYVDGVEVHNAKTKPREEQFNSTYRVVSVLTVLHQDWLNGKEYKCKVSNKGLPSSIEKTISKAKGQPREPQVYTLPPSQEEMTKNQVSLTCLVKGFYPSDIAVEWESNGQPENNYKTTPPVLDSDGSFFLYSRLTVDKSRWQEGNVFSCSVMHEALHNHYTQKSLSLSLGK

SEQ ID NO: 24 - protein, 484 aa, Artificial Sequence
  C2-4B-Fc
EVQLVESGGGLVQPGRSLRLSCAASGFTVSDYYMNWFRQAPGKGLEWVSYISSSASGSTIYYADSVKGRFTISRDNANNSLYLHMDSLRAEDTAIYFCARVVPAGSGWRWFDPWGQGTLVTVSSGGGGSGGGGSGGGGSQSVLIQPPSVSGSPGQSVTISCTGISSDVGAYDYVSWYQQHPGKVPKLMIYEVSKRPSGVPDRFSGSKSGDTASLTISGLQAEDEADYYCSSHAGSNNFYVFGTGTKLTVLGGGGSESKYGPPCPPCPAPEFLGGPSVFLFPPKPKDTLMISRTPEVTCVVVDVSQEDPEVQFNWYVDGVEVHNAKTKPREEQFNSTYRVVSVLTVLHQDWLNGKEYKCKVSNKGLPSSIEKTISKAKGQPREPQVYTLPPSQEEMTKNQVSLTCLVKGFYPSDIAVEWESNGQPENNYKTTPPVLDSDGSFFLYSRLTVDKSRWQEGNVFSCSVMHEALHNHYTQKSLSLSLGK

SEQ ID NO: 25 - protein, 484 aa, Artificial Sequence
  C2-4C-Fc
EVQLVESGGGLVQPGGSLRLSCAASGFTVSDYYMNWIRQAPGKGLEWVSYISSSASGSTIYYADSVKGRFTISRDNAKNSLYLQMNSLRAEDTAIYFCARVVPAGSGWRWFDPWGQGTLVTVSSGGGGSGGGGSGGGGSQSVLIQPPSASGSPGQSVTISCTGISSDVGAYDYVSWYQQHPGKVPKLMIYEVSKRPSGVPDRFSGSKSGNTASLTVSGLQAEDEADYYCSSHAGSNNFYVFGTGTKLTVLGGGGSESKYGPPCPPCPAPEFLGGPSVFLFPPKPKDTLMISRTPEVTCVVVDVSQEDPEVQFNWYVDGVEVHNAKTKPREEQFNSTYRVVSVLTVLHQDWLNGKEYKCKVSNKGLPSSIEKTISKAKGQPREPQVYTLPPSQEEMTKNQVSLTCLVKGFYPSDIAVEWESNGQPENNYKTTPPVLDSDGSFFLYSRLTVDKSRWQEGNVFSCSVMHEALHNHYTQKSLSLSLGK

SEQ ID NO: 26 - protein, 484 aa, Artificial Sequence
  C2-5A-Fc
EVQLVESGGGLVQPGRSLRLSCAASGFTVSDYYMNWIRQAPGKGLEWVSYISSSASGSTIYYADSVKGRFTISRDNAKNSLYLHMDSLRAEDTAIYFCARVVPAGSGWRWFDPWGQGTLVTVSSGGGGSGGGGSGGGGSQSVLIQPPSVSGSPGQSVTISCTGISSDVGAYDYVSWYQQHPGKVPKLMIYEVSKRPSGVPDRFSGSKSGNTASLTISGLQAEDEADYYCSSHAGSNNFYVFGTGTKLTVLGGGGSESKYGPPCPPCPAPEFLGGPSVFLFPPKPKDTLMISRTPEVTCVVVDVSQEDPEVQFNWYVDGVEVHNAKTKPREEQFNSTYRVVSVLTVLHQDWLNGKEYKCKVSNKGLPSSIEKTISKAKGQPREPQVYTLPPSQEEMTKNQVSLTCLVKGFYPSDIAVEWESNGQPENNYKTTPPVLDSDGSFFLYSRLTVDKSRWQEGNVFSCSVMHEALHNHYTQKSLSLSLGK

SEQ ID NO: 27 - protein, 484 aa, Artificial Sequence
  C2-5B-Fc
EVQLVESGGGLVQPGGSLRLSCAASGFTVSDYYMNWIRQAPGKGLEWVSYISSSASGSTIYYADSVKGRFTISRDNAKNSLYLQMNSLRAEDTAIYFCARVVPAGSGWRWFDPWGQGTLVTVSSGGGGSGGGGSGGGGSQSVLIQPPSASGSPGQSVTISCTGISSDVGAYDYVSWYQQHPGKVPKLMIYEVSKRPSGVPDRFSGSKSGNTASLTISGLQAEDEADYYCSSHAGSNNFYVFGTGTKLTVLGGGGSESKYGPPCPPCPAPEFLGGPSVFLFPPKPKDTLMISRTPEVTCVVVDVSQEDPEVQFNWYVDGVEVHNAKTKPREEQFNSTYRVVSVLTVLHQDWLNGKEYKCKVSNKGLPSSIEKTISKAKGQPREPQVYTLPPSQEEMTKNQVSLTCLVKGFYPSDIAVEWESNGQPENNYKTTPPVLDSDGSFFLYSRLTVDKSRWQEGNVFSCSVMHEALHNHYTQKSLSLSLGK

SEQ ID NO: 28 - protein, 484 aa, Artificial Sequence
  C2-5C-Fc
EVQLVESGGGLVQPGRSLRLSCAASGFTVSDYYMNWFRQAPGKGLEWVSYISSSASGSTIYYADSVKGRFTISRDNANNSLYLHMDSLRAEDTAIYYCARVVPAGSGWRWFDPWGQGTLVTVSSGGGGSGGGGSGGGGSQSVLIQPPSVSGSPGQSVTISCTGISSDVGAYDYVSWYQQHPGKVPKLMIYEVSKRPSGVPDRFSGSKSGDTASLTISGLQAEDEADYYCSSHAGSNNFYVFGTGTKLTVLGGGGSESKYGPPCPPCPAPEFLGGPSVFLFPPKPKDTLMISRTPEVTCVVVDVSQEDPEVQFNWYVDGVEVHNAKTKPREEQFNSTYRVVSVLTVLHQDWLNGKEYKCKVSNKGLPSSIEKTISKAKGQPREPQVYTLPPSQEEMTKNQVSLTCLVKGFYPSDIAVEWESNGQPENNYKTTPPVLDSDGSFFLYSRLTVDKSRWQEGNVFSCSVMHEALHNHYTQKSLSLSLGK

SEQ ID NO: 29 - protein, 484 aa, Artificial Sequence
  C2-6A-Fc
EVQLVESGGGLVQPGGSLRLSCAASGFTVSDYYMNWIRQAPGKGLEWVSYISSSASGSTIYYADSVKGRFTISRDNAKNSLYLQMNSLRAEDTAIYFCARVVPAGSGWRWFDPWGQGTLVTVSSGGGGSGGGGSGGGGSQSVLIQPPSVSGSPGQSVTISCTGISSDVGAYDYVSWYQQHPGKVPKLMIYEVSKRPSGVPDRFSGSKSGNTASLTISGLQAEDEADYYCSSHAGSNNFYVFGTGTKLTVLGGGGSESKYGPPCPPCPAPEFLGGPSVFLFPPKPKDTLMISRTPEVTCVVVDVSQEDPEVQFNWYVDGVEVHNAKTKPREEQFNSTYRVVSVLTVLHQDWLNGKEYKCKVSNKGLPSSIEKTISKAKGQPREPQVYTLPPSQEEMTKNQVSLTCLVKGFYPSDIAVEWESNGQPENNYKTTPPVLDSDGSFFLYSRLTVDKSRWQEGNVFSCSVMHEALHNHYTQKSLSLSLGK

SEQ ID NO: 30 - protein, 484 aa, Artificial Sequence
  C2-6B-Fc
EVQLVESGGGLVKPGGSLRLSCAASGFTVSDYYMNWIRQAPGKGLEWVSYISSSASGSTIYYADSVKGRFTISRDNAKNSLYLQMNSLRAEDTAIYFCARVVPAGSGWRWFDPWGQGTLVTVSSGGGGSGGGGSGGGGSQSVLIQPPSVSGSPGQSVTISCTGISSDVGAYDYVSWYQQHPGKVPKLMIYEVSKRPSGVPDRFSGSKSGNTASLTVSGLQAEDEADYYCSSHAGSNNFYVFGTGTKLTVLGGGGSESKYGPPCPPCPAPEFLGGPSVFLFPPKPKDTLMISRTPEVTCVVVDVSQEDPEVQFNWYVDGVEVHNAKTKPREEQFNSTYRVVSVLTVLHQDWLNGKEYKCKVSNKGLPSSIEKTISKAKGQPREPQVYTLPPSQEEMTKNQVSLTCLVKGFYPSDIAVEWESNGQPENNYKTTPPVLDSDGSFFLYSRLTVDKSRWQEGNVFSCSVMHEALHNHYTQKSLSLSLGK

SEQ ID NO: 31 - protein, 484 aa, Artificial Sequence
  C2-7A-Fc
EVQLVESGGGLVKPGGSLRLSCAASGFTVSDYYMNWIRQAPGKGLEWVSYISSSASGSTIYYADSVKGRFTISRDNAKNSLYLHMDSLRAEDTAIYFCARVVPAGSGWRWFDPWGQGTLVTVSSGGGGSGGGGSGGGGSQSALIQPPSVSGSPGQSVTISCTGISSDVGAYDYVSWYQQHPGTVPKLMIYEVSKRPSGVPDRFSGSKSGNTASLTISGLQAEDEADYYCSSHAGSNNFYVFGTGTKLTVLGGGGSESKYGPPCPPCPAPEFLGGPSVFLFPPKPKDTLMISRTPEVTCVVVDVSQEDPEVQFNWYVDGVEVHNAKTKPREEQFNSTYRVVSVLTVLHQDWLNGKEYKCKVSNKGLPSSIEKTISKAKGQPREPQVYTLPPSQEEMTKNQVSLTCLVKGFYPSDIAVEWESNGQPENNYKTTPPVLDSDGSFFLYSRLTVDKSRWQEGNVFSCSVMHEALHNHYTQKSLSLSLGK

SEQ ID NO: 32 - protein, 484 aa, Artificial Sequence
  C2-7B-Fc
EVQLVESGGGLVKPGGSLRLSCAASGFTVSDYYMNWIRQAPGKGLEWVSYISSSASGSTIYYADSVKGRFTISRDNANNSLYLQMNSLRTEDTAIYYCARVVPAGSGWRWFDPWGQGTLVTVSSGGGGSGGGGSGGGGSQSVLIQPPSVSGSPGQSVTISCTGISSDVGAYDYVSWYQQHPGKVPKLMIYEVSKRPSGVPDRFSGSKSGDTASLTISGLQAEDEADYYCSSHAGSNNFYVFGTGTKLTVLGGGGSESKYGPPCPPCPAPEFLGGPSVFLFPPKPKDTLMISRTPEVTCVVVDVSQEDPEVQFNWYVDGVEVHNAKTKPREEQFNSTYRVVSVLTVLHQDWLNGKEYKCKVSNKGLPSSIEKTISKAKGQPREPQVYTLPPSQEEMTKNQVSLTCLVKGFYPSDIAVEWESNGQPENNYKTTPPVLDSDGSFFLYSRLTVDKSRWQEGNVFSCSVMHEALHNHYTQKSLSLSLGK

SEQ ID NO: 33 - protein, 484 aa, Artificial Sequence
  C2-7BN78K-Fc
EVQLVESGGGLVKPGGSLRLSCAASGFTVSDYYMNWIRQAPGKGLEWVSYISSSASGSTIYYADSVKGRFTISRDNAKNSLYLQMNSLRTEDTAIYYCARVVPAGSGWRWFDPWGQGTLVTVSSGGGGSGGGGSGGGGSQSVLIQPPSVSGSPGQSVTISCTGISSDVGAYDYVSWYQQHPGKVPKLMIYEVSKRPSGVPDRFSGSKSGDTASLTISGLQAEDEADYYCSSHAGSNNFYVFGTGTKLTVLGGGGSESKYGPPCPPCPAPEFLGGPSVFLFPPKPKDTLMISRTPEVTCVVVDVSQEDPEVQFNWYVDGVEVHNAKTKPREEQFNSTYRVVSVLTVLHQDWLNGKEYKCKVSNKGLPSSIEKTISKAKGQPREPQVYTLPPSQEEMTKNQVSLTCLVKGFYPSDIAVEWESNGQPENNYKTTPPVLDSDGSFFLYSRLTVDKSRWQEGNVFSCSVMHEALHNHYTQKSLSLSLGK

SEQ ID NO: 34 - protein, 229 aa, Artificial Sequence
  Fc
ESKYGPPCPPCPAPEFLGGPSVFLFPPKPKDTLMISRTPEVTCVVVDVSQEDPEVQFNWYVDGVEVHNAKTKPREEQFNSTYRVVSVLTVLHQDWLNGKEYKCKVSNKGLPSSIEKTISKAKGQPREPQVYTLPPSQEEMTKNQVSLTCLVKGFYPSDIAVEWESNGQPENNYKTTPPVLDSDGSFFLYSRLTVDKSRWQEGNVFSCSVMHEALHNHYTQKSLSLSLGK

SEQ ID NO: 35 - protein, 15 aa, Artificial Sequence
  Linking peptide 1st-(G4S)3
GGGGSGGGGSGGGGS

SEQ ID NO: 36 - protein, 5 aa, Artificial Sequence
  Linking peptide 2nd-G4S
GGGGS